European Patent Application EP 4 509 186 A2, published February 19, 2025. Title: Anti-PD1 monoclonal antibody, pharmaceutical composition thereof and use thereof. Applicant: Akeso Biopharma, Inc. The sequence listing filed with the application follows.

SEQUENCE LISTING (14 sequences)

SEQ ID NO: 1 - DNA, 354 bp, synthetic construct
  misc_feature 1..354: note = Nucleotide sequence of monoclonal antibody 14C12 heavy chain variable region
  source 1..354: mol_type = other DNA
gaggtcaaactggtggagagcggcggcgggctggtgaagcccggcgggtcactgaaactgagctgcgccgcttccggcttcgcctttagctcctacgacatgtcatgggtgaggcagacccctgagaagcgcctggaatgggtcgctactatcagcggaggcgggcgatacacctactatcctgactctgtcaaagggagattcacaattagtcgggataacgccagaaatactctgtatctgcagatgtctagtctgcggtccgaggatacagctctgtactattgtgcaaaccggtacggcgaagcatggtttgcctattggggacagggcaccctggtgacagtctctgcc

SEQ ID NO: 2 - protein, 118 aa, synthetic construct
  REGION 1..118: note = The amino acid sequence of monoclonal antibody 14C12 heavy chain variable region
EVKLVESGGGLVKPGGSLKLSCAASGFAFSSYDMSWVRQTPEKRLEWVATISGGGRYTYYPDSVKGRFTISRDNARNTLYLQMSSLRSEDTALYYCANRYGEAWFAYWGQGTLVTVSA

SEQ ID NO: 3 - DNA, 318 bp, synthetic construct
  misc_feature 1..318: note = Nucleotide sequence of monoclonal antibody 14C12 light chain variable region
  source 1..318: mol_type = other DNA
gacattaagatgacacagtccccttcctcaatgtacgctagcctgggcgagcgagtgaccttcacatgcaaagcatcccaggacatcaacacatacctgtcttggtttcagcagaagccaggcaaaagccccaagaccctgatctaccgggccaatagactggtggacggggtccccagcagattctccggatctggcagtgggcaggattactccctgaccatcagctccctggagtatgaagacatgggcatctactattgcctgcagtatgatgagttccctctgacctttggagcaggcacaaaactggaactg

SEQ ID NO: 4 - protein, 106 aa, synthetic construct
  REGION 1..106: note = The amino acid sequence of monoclonal antibody 14C12 light chain variable region
DIKMTQSPSSMYASLGERVTFTCKASQDINTYLSWFQQKPGKSPKTLIYRANRLVDGVPSRFSGSGSGQDYSLTISSLEYEDMGIYYCLQYDEFPLTFGAGTKLEL

SEQ ID NO: 5 - DNA, 354 bp, synthetic construct
  misc_feature 1..354: note = Nucleotide sequence of monoclonal antibody 14C12H1L1 heavy chain variable region
  source 1..354: mol_type = other DNA
gaagtgcagctggtcgagtctgggggagggctggtgcagcccggcgggtcactgcgactgagctgcgcagcttccggattcgcctttagctcctacgacatgtcctgggtgcgacaggcaccaggaaagggactggattgggtcgctactatctcaggaggcgggagatacacctactatcctgacagcgtcaagggccggttcacaatctctagagataacagtaagaacaatctgtatctgcagatgaacagcctgagggctgaggacaccgcactgtactattgtgccaaccgctacggggaagcatggtttgcctattgggggcagggaaccctggtgacagtctctagt

SEQ ID NO: 6 - protein, 118 aa, synthetic construct
  REGION 1..118: note = The amino acid sequence of monoclonal antibody 14C12H1L1 heavy chain variable region
EVQLVESGGGLVQPGGSLRLSCAASGFAFSSYDMSWVRQAPGKGLDWVATISGGGRYTYYPDSVKGRFTISRDNSKNNLYLQMNSLRAEDTALYYCANRYGEAWFAYWGQGTLVTVSS

SEQ ID NO: 7 - DNA, 321 bp, synthetic construct
  misc_feature 1..321: note = Nucleotide sequence of monoclonal antibody 14C12H1L1 light chain variable region
  source 1..321: mol_type = other DNA
gacattcagatgactcagagcccctcctccatgtccgcctctgtgggcgacagggtcaccttcacatgccgcgctagtcaggatatcaacacctacctgagctggtttcagcagaagccagggaaaagccccaagacactgatctaccgggctaatagactggtgtctggagtcccaagtcggttcagtggctcagggagcggacaggactacactctgaccatcagctccctgcagcctgaggacatggcaacctactattgcctgcagtatgatgagttcccactgacctttggcgccgggacaaaactggagctgaag

SEQ ID NO: 8 - protein, 107 aa, synthetic construct
  REGION 1..107: note = The amino acid sequence of monoclonal antibody 14C12H1L1 light chain variable region
DIQMTQSPSSMSASVGDRVTFTCRASQDINTYLSWFQQKPGKSPKTLIYRANRLVSGVPSRFSGSGSGQDYTLTISSLQPEDMATYYCLQYDEFPLTFGAGTKLELK

SEQ ID NO: 9 - protein, 8 aa, synthetic construct
  REGION 1..8: note = HCDR
GFAFSSYD

SEQ ID NO: 10 - protein, 8 aa, synthetic construct
  REGION 1..8: note = HCDR
ISGGGRYT

SEQ ID NO: 11 - protein, 11 aa, synthetic construct
  REGION 1..11: note = HCDR
ANRYGEAWFAY

SEQ ID NO: 12 - protein, 6 aa, LCDR
QDINTY

SEQ ID NO: 13 - skipped

SEQ ID NO: 14 - protein, 9 aa, synthetic construct
  REGION 1..9: note = LCDR
LQYDEFPLT